European Patent Specification EP 3 971 284 B1, published November 8, 2023. Title: MODIFIED NATURAL KILLER CELLS AND NATURAL KILLER CELL LINES HAVING INCREASED CYTOTOXICITY. Applicant: Onkimmune Limited. The sequence listing filed with the application follows.

SEQUENCE LISTING (12 sequences)

SEQ ID NO: 1 - DNA, 9540 bp, Homo sapiens
ctctggcctctgttctttcttgtgagtccgtctacacttggggtttccacatgtctttttctgctcatgaccttgatactctgggtatttcagaaatgctacacatacgtttctccattacggtcagatgtgacatcttgagtggactcatcaatcacctacagaatgtggagtccaacagcaagatcctctcacgtcccaaagcctcaggtcttaccctggtctggaaatcaagcacaaatgagcccctcccaatgtcccaggcaccactgaccccacaaccactgtgacgagtgggattcatgacaacaatctgcaaaggaagaaactgaggctcagtgatgggacattacaaaccaaggtcacgtaggcagcggatgataaccagtcatcaaataaatatcaactccctcccccactccccaaatcaaagctcaaacataagtcattgttcccaaaatgttgaccaggaattgaggtgcagagggacggctaaggacgcaatgggcaccgaggaggcaggaaagactcagaggtttcttcccgggggggagggagtggacgctggagcaaaaacatttaaaaaggggaagttaagaggggactatttggttgaaagaaaacccacaatccagtgtcaagaaagaagtcaacttttcttcccctacttccctgcatttctcctctgtgctcactgccacacacagctcaacctggacagcacagccagaggcgagatgcttctctgctgatctgagtctgcctgcagcatggacctgggtcttccctgaagcatctccagggctggagggacgactgccatggtaaggaccccacaacgctgtgctgatggatgggctgaaggagggagggtgaccatgtgggaagctgtgagaaggaaggggaagccactgctaccctcatcaggaagggcagacacaagaagcaccagttctatttgctgctacatcccggctctcggtgagacgaggagaaaccagacagacagtggctgggggtcaggaaagaccccattacagtctgaaatgtctgcagagggcccagtgcctgcccccacctcagctctaaaagaatgagagtcaggctcctgggagggcagttccgcttcttgtgtggctgcagatgacaacaccccatgagaaggacccagcctctgagtgtccacacagggtgggaaggaggggaggctatttctctctgtgtgtctctgtcccgccagcaccgagggctcatccatccgcagagcagggcagtgggaggagacgccatgacccccatcgtcacagtcctgatctgtctcggtgagatttgaagagagaggggagcttctaacctaggagggacctcaccccacagccaaactctggtccctaaggagaccccaggggctcacaaagatcccagggaggggaggacctgctcaggcttcagggggcaaatccctcacagggaactctcttccagggctgagtctgggccccaggacccgcgtgcagacaggtgagtctgtccccagctctcccaggtccctcctcctcactggggacaaggggccacctccgtgcagctggggatggggattagaagttctggactgactgatgggggcatctggagggtcctgggctgagagctgagatctgttgggtgggaaatgacttcgaatctgacctttgatttccttccagggaccatccccaagcccaccctgtgggctgagccagactctgtgatcacccaggggagtcccgtcaccctcagttgtcaggggagccttgaagcccaggagtaccgtctatatagggagaaaaaatcagcatcttggattacacggatacgaccagagcttgtgaagaacggccagttccacatcccatccatcacctgggaacacacagggcgatatggctgtcagtattacagccgcgctcggtggtctgagctcagtgaccccctggtgctggtgatgacaggtgagaggacactcagggatcccagccccaggctctgccctcaggaaggaggctctcaggggtgtctccctctcacagcccagccctggggatgatgtgggaggtgggagccccatttaacacgatgcctccttctctcctaggagcctacccaaaacccaccctctcagcccagcccagccctgtggtgacctcaggaggaagggtgaccctccagtgtgagtcacaggtggcatttggcggcttcattctgtgtaaggaaggagaagatgaacacccacaatgcctgaactcccagccccatgcccgtgggtcgtcccgcgccatcttctccgtgggccccgtgagcccgaatcgcaggtggtcgcacaggtgctatggttatgacttgaactctccctatgtgtggtcttcacccagtgatctcctggagctcctggtcccaggtgagaaattcacagcattgtctggagttccctgagtctccctgagtctccaggcaggtggggagcagccgtgtctcagggcagttccaggtgggatgatgttggggcgagagggctcaggggtcctggggccagagacacaggaagatcagcagtggtgaggcaccgggggagagggagggtttgtggggaagcctgagggtcggctcctggaaaccatgagcaccttttcccaggtgtttctaagaagccatcactctcagtgcagccgggtcctgtcatggcccctggggaaagcctgaccctccagtgtgtctctgatgtcggctatgacagatttgttctgtacaaggagggggaacgtgaccttcgccagctccctggccggcagccccaggctgggctctcccaggccaacttcaccctgggccctgtgagccgctcctacgggggccagtacagatgctacggtgcacacaacctctcctctgagtgctcggcccccagcgaccccctggacatcctgatcacaggtgaggagcccagcgggttcagtcagggacccagactctgcacaggccctgccgggggaatccaattagtgatggccaggatgaggcggggggtggtcccaagggagggagagacagagagagagacaggggatgggtggggaggggaagactcagagaaaacagagacagaggctcctagagaggcctggggaggtctcagctcagagcaaggtggggcagcccctcacccatccttcttctctccaggacagatccgtggcacacccttcatctcagtgcagccaggccccacagtggcctcaggagagaacgtgaccctgctgtgtcagtcatggcggcagttccacactttccttctgaccaaggcgggagcagctgatgccccactccgtctaagatcaatacacgaatatcctaagtaccaggctgaattccccatgagtcctgtgacctcagcccacgcggggacctacaggtgctacggctcactcaactccgacccctacctgctgtctcaccccagtgagcccctggagctcgtggtctcaggtgggggccttgaccctgtcctctctgagctcaaaggctcagctcaggccctgccccccaggagagctctgggctgggatggagtgagcgggggtctgagcggggctcagccagtgggagactcaccctcagagggaaggaggacaacaggccctcccaggcctgcgcacactcagcggcatcgccagcatcatggacaggagaggcgggtggagggaggggcctggggaggccacagggcccatgtagagaaatttggtttgaggtggagacttcaggaaagccccagctcctcaccctcctctcattctttcacccaggaccctccatgggttccagccccccacccaccggtcccatctccacacctggtgagtccctgaggcctctggctcgaagggagcgcagcgacccccagggcagctttgagtgtccaggaggatcccattcccttcagggactcaatcaagggcttctgtccagggagctgggcagagccagaggaggggccacagggtccccagggctctgaggctgggctggtgaggggtggggggtcaaggcagagagaaatgttggggcccagcctgggggaggagcagccgggctgatgtggggagcagggcagccccagccctcacctccccgtcctgacccagcaggccctgaggaccagcccctcacccccactgggtcggatccccaaagtggtgagtgaggggctctgagtgggaggtgggcggggtcccggggaggcaggggtgggttctgtcctaggttcaggctcctctggaggtggtgatgtagacaggctcctcccctgcctgggcctcagtttctccaagtgtaaaggagagaggcctgcaggtgggaaagttcctttcagctctcactcccagctgtgacctcctgggagaggaggcccctcagggaagactccaagactcgattccgcgggggcctgtcccgtcccacctgcagcagagacggtgacctggggcaggggaggggagcagagtcgtggttcaggacggtaaggctctttccctgcagctccggggctcggctctggtgcaggaacaagggctgcaggtcagactcccaggctcccttcccagctctgccgcttcctggctgggggcccggggcaggcgattcccctctctgagcgtcagtttttcatctgtagagtgggtggggtggatgtttgtgtgctgcacgactgttgtgggggttggaggtggtgaacagaaggtccagcagtcacctgcacacagtaggcgctcatttcaatgacatcacccccatccctgacatcatcgtgctcaaggtctgggaaggcacctgggggttgtgatcggcatcttggtggccgtcgtcctactgctcctcctcctcctcctcctcttcctcatcctccgacatcgacgtcagggcaaacactggacatcgagtgagtagggaaggggaaaccctgtgggccgaccgagggtgggctcagggcacagccaaagagaatccaaaccactgggcaaatgcagctttgagaaactgttccagcatttctcaccaggtgaatggagaaagcacttaacgtcagtcccatctacaaatataaagtgtcctccgggctcagtcccatctacaaatgtaaagtgtccttcggactctgtccatctcatgaggcatttggaacatggaggcaggagtgtttttaggtttccttccttaccttcgagctgtgtgtgcagggcagggggctccaatgttcccagggctgaggctctgtccttcttcccccagcccagagaaaggctgatttccaacatcctgcaggggctgtggggccagagcccacagacagaggcctgcagtggaggtaattctgcccgaagaccccagactcccacctgctcgtggcccatacactgcccctaaagctcccattcctcccccaggtccagcccagctgccgacgcccaggaagaaaacctctgtgagtgagaggaagaggtgaccagccaggagggagataggggccccgaagtttccgtagcaatggggaaaggggcaccggctggaaagggtctggggctcagggtgagatcatctcaccccacactgtgggacctcagggacattgcagcccctccctgcatctcagtagccccatctgggagcagggcaggggctggcaggactcagaggtcccagggaaccttcccaagagacgaaccccttgctctgccccagcagatgctgccgtgaaggacacacagcctgaagatggggtggagatggacactcgggtgagaccccgcccctgtcccaggcaccaaaggcctcctggtgccagatctaatccagcaggacttctctgtcctccttcccccggctctcagcatcgtcacggtggacccctccttgtccagcacgctgcctcccgcctgctgtgacctcactctctcctgctgtcctgggacctcgtgggcctcctcccgggtccccttcctgctcctcatcctctgtttggccgtctggttgttagagcgctccccaggcctctggaggatgaggaataaatgaaccaccccggtcccctgggctccccttcattcattcaaccagtgagtgttcccagggagctcactgtggatcaggctccccatgggagctgcagacacagcagggagcaaagccgcccccgcctcctgagctcacctcatggtgggagacaaaatgcaaataaatgcgccatgtccaggagtgcaacgtgcttaaaggaacatacaccagggaaagggcagagagtgtggggcagtggggccagtctgaatggaaggggagggctgtctgctcagctgtcatctgagaagcctggacagagtggggcacacgatcctctaatggacgagcccctgcaggcagaggaaacagccgtgcaaaggccccgaggcagcagcgagctcttgcgggaaggcccatgaggctgcagccaaatgggcaaggtcaaagtgaggagcagaggccagaaccacaggaagggagcggccagaccctccacggccttagggcgtccctgagattccatcgggaaagggatgtaatcggatcaccccgggaacagtgaggaaaattgactccaggaggtcagggggactcaaggacaccccccaccactgtctctctccagcagagcccacatgatgaagacccccaggcagtgacatatgccccggtgaaacactccagacctaggagagaaatggcctctcctccctccccactgtccggggaattcctggacacaaaggacagacaggcagaagaggacagacagatggacactgagagagtcctttcctctccaggcccccaggcctcccccacccccaccacgttccttacctctcactctcccccgctgcaggctgctgcatctgaagccccccaggatgtgacctacgcccagctgcacagcttgaccctcagacggaaggcaactgagcctcctccatcccaggaaagggaacctccagctgagcccagcatctacgccaccctggccatccactagcccggagggtacgcagactccacactcagtagaaggagactcaggactgctgaaggcacgggagctgcccccagtggacaccaatgaaccccagtcagcctggacccctaacaaagaccatgaggagatgctgggaactttgggactcacttgattctgcagtcgaaataactaatatccctacattttttaattaaagcaacagacttctcaataatcaatgagttaaccgagaaaactaaaatcagaagtaagaatgtgctttaaactgaatcacaatataaatattacacatcacacaatgaaattgaaaaagtacaaaccacaaatgaaaaaagtagaaacgaaaaaaaaaaactaggaaatgaatgacgttggctttcgtataaggaatttagaaaaagaataaccaattattccaaatgaaggtgtaagaaagggaataagaagaagaagagttgctcatgaggaaaaaccaaaacttgaaaattcaacaaagccaatgaagctcattcttgaaaatattaattacagtcataaatcctaactacattgagcaagagaaagaaagagcaggcacgcatttccatatgggagtgagccagcagacagcccagcagatcctacacacattttcacaaactaaccccagaacaggctgcaaacctataccaatatactagaaaatgcagattaaatggatgaaatattcaaaactggagtttacataatgaacgtaagagtaatcagagaatctgactcattttaaatgtgtgtgtatgtgtgtgtatatatatgtgtgtgtgtgtgtgtgtgtgtgtgtgtgaaaaacattgactgtaataaaaatgttcccatcgtatcaactccagttcaggaagtttcactggtgatttcttacaaatattgacgcactaatgaaacacacaaacacacccagagcatcacaaatgtttcttgagaatagaaaaagaggcaatgtgcccgggtgcggtggctcacgcctgtaatctcaacacctagggaggcagaggccacagattacttgaggccgggagttcaagaccagcatggccaacaaggcaaaaccccatctctactaaaaatacaaaaattagctggacatggtggcgcacgctgcaatcccagctacttgggaggcagaggcaggaggatcacttgaatgaacccgggaggtggaggttgaagtgagcaaaaacaaaccccctacaattcagcctaggatatgtttattaaatttacatttgtctttttgcttaagattgctttggtattcatcctctttttggttccatatgaattttaggatttttttctaattctgtgaaaaaaatgatgttgatattttgatgggaattgcattgaacctaaatattgctttgggaagtgtgatcattttcacaatattgattctgccaatccatgagcatgggatatatttctattttgctgtgtcatctacgatttctttctgcagcattttgttgttcttcttgtagagatctttcacctcctcagttaggtatattcttagatatttttaattttttgcaactgatgtacaagggattgagttttgcagcaacctggatgagctggaggccattattcatgacaccacatccagctaatttttgtatttcttgtagagatgaggttttgccatgttgcccaggctggtcttgaactcctgggcccaagtgacccgcccgccttgacctcccaaagtgctgggactgcaggcatgagccacggtgcctggcccatcatagcacttttgatcattaggataattccttctccttgtcatttttggacacatgcttcccacatgcctcatcttccagagagggtttccaccagggctgtgctgggagttaaggctggaaaaggggagatggttccacctgccagtgccacatgagtctactcagggctgtaaccagcagggagggtccagtgtgagcctcagactcgcatgtgggacagacgcccatgtgtgacaacgctgcagtgaatctgtttcacacacatggaggaggcggctcagggctgaccatggacctgagtcaatgagcagagatatcccagtgccatccacaaacacaggggagaaggagccacaacttcccactttcatccaaaaccccgacccctccctgtctgtgagggccctggggttctcctctgtctcatacagaggcagaaacctcccccttagtgacccccagctttgcaagtcaccagcagcccctcggcgctggcatcttctgcttcttaaggtttcctgcctatgacaggaagtctcatttctcattttcttcattggaccatggctacatatttcagacacattataagtaggttttcccagtgttaggagcagatgtgggctgttgagcacataagtcactcac

SEQ ID NO: 2 - protein, 101 aa, Homo sapiens
GAYPKPTLSAQPSPVVTSGGRVTLQCESQVAFGGFILCKEGEDEHPQCLNSQPHARGSSRAIFSVGPVSPNRRWSHRCYGYDLNSPYVWSSPSDLLELLVP

SEQ ID NO: 3 - DNA, 23 bp, Homo sapiens
gagtcacaggtggcatttggcgg

SEQ ID NO: 4 - DNA, 23 bp, Homo sapiens
cgaatcgcaggtggtcgcacagg

SEQ ID NO: 5 - DNA, 20 bp, Homo sapiens
gggagccccatttaacacga

SEQ ID NO: 6 - DNA, 20 bp, Homo sapiens
gggagactcagggaactcca

SEQ ID NO: 7 - DNA, 7375 bp, Homo sapiens
ctttggaccttcttcaactctgttttgtctctgttgagttaaggcttttaagaacacctgaattctttccttctgcaaaaccagaggcagcttcttttccgcctattttcagtttatttcttgtgattttagtttttttctcttaaccaaatgctaaatggatttaggagaaataaacttatttgtaaagctgtcaagggaccattagaaggatggtgcttcacagatagaatacagtttttattaatgatgcctagacaaatcctgccattagcccaagggctcagaaagttagcagcctagtagttttggagttgtcaatgaaatgaattggactggatggttaaggatgcccagaagattgaataaaattgggatttaggaggacccttgtactccaggaaattctccaagtctccacttagttatccagatcctcaaagtgaacatgaagcttcagtttcaaattgaatacattttccatccatggattggcttgttttgttcagttgagtgcttgaggttgtcttttcgacgtaacagctaaacccacggcttcctttctcgtaaaaccaaaacaaaaaggctttctattcaagtgccttctgtgtgtgcacatgtgtaatacatatctgggatcaaagctatctatataaagtccttgattctgtgtgggttcaaacacatttcaaagcttcaggatcctgaaaggttttgctctacttcctgaagacctgaacaccgctcccataaagccatggcttgccttggatttcagcggcacaaggctcagctgaacctggctaccaggacctggccctgcactctcctgttttttcttctcttcatccctgtcttctgcaaaggtgagtgagacttttggagcatgaagatggaggaggtgtttctcctacctgggtttcatttgtttcagcagtcaaaggcagtgatttatagcaaagccagaagttaaaggtaaaactccaatctggcttggctggctctgtattccagggccagcagggagcagttgggcggcagcaaataaggcaaagagatagctcagaacagagcgccaggtatttagtaggggcttcatgaatgcatgtgagttggtttagtagagagacacaggcaatttcagacccttctatgagactggaagtgatttaagagggaaaggatagccatagtcctgaatacatttgagctgggtttcaggatgagctcacaagttcctttaaaaaaaattgacttaagcaaatcctgggaagagtttttttgctatacaattcaaggttttaaggtcctcggattcatatactttataaatgaattagccagcttgtttaaaatgtagggaaattgtgggaagaatgccttctttacttaattcaaggttttaaggttctcttaatcaattctactagctaattagccaattatttaaaaataaaagtttgaaattgccaaaaaaaaaagacaaggaaaaggaaagaaagaaagccaccagtctgtttggcatacaatacttaattgttgcctgacctacgtgtgggtttcagatgcagatcctcagttttcagctcttcagagactgacaccaggtttgttacacggcttaaaatgatgagtatatccattgaatctcaaccttatctctctctagaccttcttggttaagaaaccatgtagtttgtatgaagtaggtactcaaaagatatttgatgatttaatttttactggagaagaaatattcatatatgttttcttatttttacatgttttaaatatgtaaagattaaataaacactcttagaagtatttaaatttcctaaagtaaatttatctcaaccagtaacaggaccctcccaatactggaaagttgagtgtgaccgcatttagtggtgatgagtgtgagcttgcttggggagagggcaggacatttaggatttcttaagcttagagtcaatacaataaagattattgagtgctcacttgggtgggctataatcactgctcacaggagttcatgaaccacaagtaaaagagtgaggagatatgattagctcacaaataactttaatacagagcagaaagtaatgaactactgcaatggagttatcacagtgctaaggatgctcagagggcatctctgataggcagaggtgagggttagggaaggaagctgtagtctagctagctagagctgctggaatagacatgacaatggctgctgccaaactgttttctcttctgaggacagatgtcccgtgcaagtggcttggtggaagggactagtgtctctaatatagggtgatttataagcaggaaagtgtgtcctagaaattcagaccagagtgatagattggaattggatcatgggggactcattgaatgttatttattgtatttgtttttgcgatcagtgttagtaaagtgtcaaagggattgagcagatgagtgacatcatgcaacacaagttttgagtttcacttgtcagactgactggagaggggcctggttagttacaggaaggtaatttggcatgcagccactatttttgagttgatgcaagcctctctgtatggagagctggtctcctttatcctgtgggaaaagagaacaaaggagcatgggagtgttcaagggaaggagaaataaagggcagagaggcagcggtggtgtcaggggaagcccacaggagttaacagcagggttgcctcaacctagagaggaagcgacctggtgccctcggctctgtggcttccttcatctaacaacatcttccactctacaacaatgccagggaaggcggaggctggtacagtgcatcaagacacagctactcctgggtgacagaggttcagggccagctcactaagtaggcagaagtttttgacatatactttgagagataaagcaagattctgtacctcaaccttcagaatttcccctaccactcattatagttccggagctatatagctcctatcattctatcataaccttagaataccagagaacatatcatctcatctaattatctcttactatatgtgaaaaaaatgaaggacatgggggaagtgtgacttgccccaaatcacatatttcatggtagagccaggtcttctgtttgtcatatcagtgttcttcctgccacaaccatcttgaagaatctatttctcagtaagaaaatatctttatggagagtagctggaaaacagttgagagatggaggggaggctgggggtgtggagaggggaaggggtaagtgatagattcgttgaaggggggagaaaaggccgtggggatgaagctagaaggcagaagggcttgcctgggcttggccatgaaggagcatgagttcactgagttccctttggcttttccatgctagcaatgcacgtggcccagcctgctgtggtactggccagcagccgaggcatcgccagctttgtgtgtgagtatgcatctccaggcaaagccactgaggtccgggtgacagtgcttcggcaggctgacagccaggtgactgaagtctgtgcggcaacctacatgatggggaatgagttgaccttcctagatgattccatctgcacgggcacctccagtggaaatcaagtgaacctcactatccaaggactgagggccatggacacgggactctacatctgcaaggtggagctcatgtacccaccgccatactacctgggcataggcaacggaacccagatttatgtaattggtgagcaaagccatttcactgagttgacacctgttgcattgcagtcttctatgcacaaaaacagttttgttccttaatttcaggaggtttacttttaggactgtggacattctctttaagagttctgtaccacatggtagccttgcttattgtgggtggcaaccttaatagcattctgactgtaaaataaaatgatttggggaagttggggctctcgctctggagtgctaaccatcatgacgtttgatctgtacttttgatatgatatgatgctcctggggaagtagtcccaaatagccaaacctattggtgggctacccatgcaatttaggggtggacctcaaggcctggaagctctaatgtccttttttcaccaatgttggggagtagagccctagagtttaaaactgtctcagggaggctctgctttgttttctgttgcagatccagaaccgtgcccagattctgacttcctcctctggatccttgcagcagttagttcggggttgtttttttatagctttctcctcacagctgtttctttgagcaaaatggtgagtgtggtgctgatggtgcaccatgtctgatggggatacctttagtggtatcaactggccaaaagatgatgttgagtttagtgttcttgagatgagatgaggcaataaatgaagaggaaggacagtggtaaagaacgcactagaaccgtaggcattggcatttgaggtttcagaatgactaatattttagatgaatttgtttgacattgaatgttcatgtgcttctgagcagggtttcaatttgagtaaccgttgcaataacatggggcagctgttttgctctttgtcttcatgacaactgtacttaagctaacagccctgaaacatgagattaggctgggcagaatgctgctagagaggaccacttggatggtctttattctccttctccatgtccctctccatcacctggaagtcacctctgggtgccactctggtgccttccttgtcgaagctgtagctgctcacatgacacctatccctgttatccagtttgcttgactgggacgttttgccttccccttcagccaggaagtgaaagtcccagtttttatttatcacaggtgttggtattggtggtagaagaggtagaattatggaatcaggcctcctgtcaggatttctttttgacagtccctctcagacacctctgcctaaggccagctttgccattacaaactctcccttctccctctctcccttcttctcttcctcttccttcttctcgctctttctctctctctctttctccctctctgtctcttatacacatacacaaagatatactctattccaacatcctctacccaacctgacagagatgtcctttgctgtaggttcagcagtggggatgagaaatacagctctcaaacaggataactaaagcttattatcttatcaagcttgttcccttgcagacaagattgatcaattatcataggctttctgggtgttctttctgaagctttctcaaagtctctttctcctatcttccattcaaggcaaatgattgccatttaacatcaaaatcacagttatttatctaaaataaattttaatagctgaatcaagaaaatctcctgaggtttataattctgtatgctgtgaacattcatttttaaccagctagggacccaatatgtgttgagttctattatggttagaagtggcttccgtattcctcagtagtaattactgtttctttttgtgtttgacagctaaagaaaagaagccctcttacaacaggggtctatgtgaaaatgcccccaacagagccagaatgtgaaaagcaatttcagccttattttattcccatcaattgagaaaccattatgaagaagagagtccatatttcaatttccaagagctgaggcaattctaacttttttgctatccagctatttttatttgtttgtgcatttggggggaattcatctctctttaatataaagttggatgcggaacccaaattacgtgtactacaatttaaagcaaaggagtagaaagacagagctgggatgtttctgtcacatcagctccactttcagtgaaagcatcacttgggattaatatggggatgcagcattatgatgtgggtcaaggaattaagttagggaatggcacagcccaaagaaggaaaaggcagggagcgagggagaagactatattgtacacaccttatatttacgtatgagacgtttatagccgaaatgatcttttcaagttaaattttatgccttttatttcttaaacaaatgtatgattacatcaaggcttcaaaaatactcacatggctatgttttagccagtgatgctaaaggttgtattgcatatatacatatatatatatatatatatatatatatatatatatatatatatatatatatatattttaatttgatagtattgtgcatagagccacgtatgtttttgtgtatttgttaatggtttgaatataaacactatatggcagtgtctttccaccttgggtcccagggaagttttgtggaggagctcaggacactaatacaccaggtagaacacaaggtcatttgctaactagcttggaaactggatgaggtcatagcagtgcttgattgcgtggaattgtgctgagttggtgttgacatgtgctttggggcttttacaccagttcctttcaatggtttgcaaggaagccacagctggtggtatctgagttgacttgacagaacactgtcttgaagacaatggcttactccaggagacccacaggtatgaccttctaggaagctccagttcgatgggcccaattcttacaaacatgtggttaatgccatggacagaagaaggcagcaggtggcagaatggggtgcatgaaggtttctgaaaattaacactgcttgtgtttttaactcaatattttccatgaaaatgcaacaacatgtataatatttttaattaaataaaaatctgtggtggtcgttttccggagttgtctttatcatccttgcatttgaatattgtgttcaaatttttgattgattcattcagtatctggtggagtctccaatattagaaatactggaaacaaactgaaaaaccacaaaaggacaaataatgcttcatgagtcagctttgcaccagccattacctgcaagtcattcttggaaggtatccatcctctttccttttgatttcttcaccactatttgggatataacgtgggttaacacagacatagcagtcctttataaatcaattggcatgctgtttaacacaggttcttcacctcccctttcttaccgcctgctttctcagctcaactatcacaggcattacagttgtcatggcaaccccaatgttggcaaccacgtcccttgcagccattttgatctgccttcctgaaatatagagcttttccctgtggcttccaaatgaactattttgcaaatgtggggaaaacacacacctgtggtcctatgttgctatcagctggcacacctaggcctggcacactaagccctctgtgattcttgcttaaccaatgtatagtctcagcacatttggtttccacttaaggtttcct

SEQ ID NO: 8 - protein, 36 aa, Homo sapiens
MACLGFQRHKAQLNLATRTWPCTLLFFLLFIPVFCK

SEQ ID NO: 9 - DNA, 23 bp, Homo sapiens
cactcacctttgcagaagacagg

SEQ ID NO: 10 - DNA, 23 bp, Homo sapiens
ccttgtgccgctgaaatccaagg

SEQ ID NO: 11 - DNA, 29 bp, Homo sapiens
aggacccttgtactccaggaaattctcca

SEQ ID NO: 12 - DNA, 26 bp, Homo sapiens
agcccctactaaatacctggcgctct